European Patent Specification EP 3 342 422 B1, published June 19, 2024. Title: TILAPIA LAKE VIRUS VACCINES. Applicant: THE STATE OF ISRAEL, MINISTRY OF AGRICULTURE & RURAL DEVELOPMENT, KIMRON VETERINARY INSTITUTE RAMOT AT TEL-AVIV UNIVERSITY LTD. Application EP 15749196.0. The sequence listing filed with the application follows.

SEQUENCE LISTING (5 sequences)

SEQ ID NO: 1 - DNA, 20 bp, Artificial Sequence
  PCR forward primer
gttgggcacaaggcatccta

SEQ ID NO: 2 - DNA, 23 bp, Artificial Sequence
  PCR reverse primer
tatcacgtgcgtactcgttcagt

SEQ ID NO: 3 - DNA, 15 bp, Artificial Sequence
  FAM probe
agggaacggctattg

SEQ ID NO: 4 - DNA, 22 bp, Artificial Sequence
  Reverse primer
gggtcagaaagacagctacgtt

SEQ ID NO: 5 - DNA, 22 bp, Artificial Sequence
  Forward primer
ctcagctcgttgtagaaggtgt